European Patent Specification EP 4 074 823 B1, published December 25, 2024. Title: DETECTION METHOD. Applicant: Toppan Printing Co., Ltd. The sequence listing filed with the application follows.

SEQUENCE LISTING (7 sequences)

SEQ ID NO: 1 - DNA, 24 bp, Artificial Sequence
  synthesized oligonucleotide sequence
cgcgccgaggcgcagctcatgccc

SEQ ID NO: 2 - DNA, 31 bp, Artificial Sequence
  synthesized oligonucleotide sequence
tctgcctcacctccaccgtgcarctcatcaa

SEQ ID NO: 3 - DNA, 35 bp, Artificial Sequence
  Synthesized oligonucleotide sequence
  misc_feature (1)..(1): modified with Alexa488
  misc_feature (5)..(5): modified with Black Hole Quencher
ttcttagccggttttccggctgagacctcggcgcg

SEQ ID NO: 4 - DNA, 27 bp, Artificial Sequence
  synthesized oligonucleotide sequence
acggacgcggagcaggaggcagccgaa

SEQ ID NO: 5 - DNA, 31 bp, Artificial Sequence
  synthesized oligonucleotide sequence
aatattgtctttgtgttcccggacatagtca

SEQ ID NO: 6 - DNA, 35 bp, Artificial Sequence
  synthesized oligonucleotide sequence
  misc_feature (1)..(1): modified with Redmond Red
  misc_feature (4)..(4): modified with Epoch Eclipse Quencher
  misc_feature (36)..(36): modified with hexanediol
tcttcggccttttggccgagagactccgcgtccgt

SEQ ID NO: 7 - DNA, 44 bp, Homo sapiens
gggcatgagctgcgtgatgagctgcacggtggaggtgaggcaga